European Patent Specification EP 3 796 979 B1, published June 4, 2025. Title: miR-181 inhibitors and uses thereof. Applicant: Fondazione Telethon. The sequence listing filed with the application follows.

SEQUENCE LISTING (114 sequences)

SEQ ID NO: 1 - RNA, 23 nt, Artificial Sequence
  synthetic
aacauucaacgcugucggugagu

SEQ ID NO: 2 - RNA, 23 nt, Artificial Sequence
  synthetic
aacauucauugcugucggugggu

SEQ ID NO: 3 - RNA, 22 nt, Artificial Sequence
  synthetic
aacauucaaccugucggugagu

SEQ ID NO: 4 - RNA, 23 nt, Artificial Sequence
  synthetic
aacauucauuguugucggugggu

SEQ ID NO: 5 - RNA, 7 nt, Artificial Sequence
  synthetic
acauuca

SEQ ID NO: 6 - DNA, 16 bp, Artificial Sequence
  synthetic
cgacagcgttgaatgt

SEQ ID NO: 7 - DNA, 16 bp, Artificial Sequence
  synthetic
cgacagcaatgaatgt

SEQ ID NO: 8 - DNA, 322 bp, Artificial Sequence
  synthetic
acccaccgacaatgctgaatgttcgatactcaccgacaatagtgaatgttcgatacccaccgacaatgctgaatgttcgatactcaccgacaatagtgaatgttcgatacccaccgacaatgctgaatgttcgatactcaccgacaatagtgaatgttagatctacccaccgacaatgctgaatgttcgatactcaccgacaatagtgaatgttcgatacccaccgacaatgctgaatgttcgatactcaccgacaatagtgaatgttcgatacccaccgacaatgctgaatgttcgatactcaccgacaatagtgaatgtt

SEQ ID NO: 9 - DNA, 323 bp, Artificial Sequence
  synthetic
acccaccgacaattctgaatgttcgatactcaccgacaaatgtgaatgttcgatacccaccgacaattctgaatgttcgatactcaccgacaaatgtgaatgttcgataacccaccgacaattctgaatgttcgatactcaccgacaaatgtgaatgttagatctacccaccgacaattctgaatgttcgatactcaccgacaaatgtgaatgttcgatacccaccgacaattctgaatgttcgatactcaccgacaaatgtgaatgttcgatacccaccgacaattctgaatgttcgatactcaccgacaaatgtgaatgtt

SEQ ID NO: 10 - DNA, 322 bp, Artificial Sequence
  synthetic
acccaccgacaattctgaatgttcgatactcaccgacaaatctgaatgttcgatacccaccgacaattctgaatgttcgatactcaccgacaaatctgaatgttcgatacccaccgacaattctgaatgttcgatactcaccgacaaatctgaatgttagatctacccaccgacaattctgaatgttcgatactcaccgacaaatctgaatgttcgatacccaccgacaattctgaatgttcgatactcaccgacaaatctgaatgttcgatacccaccgacaattctgaatgttcgatactcaccgacaaatctgaatgtt

SEQ ID NO: 11 - DNA, 321 bp, Artificial Sequence
  synthetic
acccaccgacaaagctgaatgttcgatactcaccgacaggtctgaatgttgatacccaccgacaaagctgaatgttcgatactcaccgacaggtctgaatgttcgatacccaccgacaaagctgaatgttcgatactcaccgacaggtctgaatgttagatctacccaccgacaaagctgaatgttcgatactcaccgacaggtctgaatgttcgatacccaccgacaaagctgaatgttcgatactcaccgacaggtctgaatgttcgatacccaccgacaaagctgaatgttcgatactcaccgacaggtctgaatgtt

SEQ ID NO: 12 - DNA, 321 bp, Artificial Sequence
  synthetic
acccaccgacaaagctgaatgttcgatactcaccgacaggtctgaatgttgatacccaccgacaaagctgaatgttcgatactcaccgacaggtctgaatgttcgatacccaccgacaaagctgaatgttcgatactcaccgacaggtctgaatgttagatctacccaccgacaattctgaatgttcgatactcaccgacaaatgtgaatgttcgatacccaccgacaattctgaatgttcgatactcaccgacaaatgtgaatgttcgatacccaccgacaattctgaatgttcgatactcaccgacaaatgtgaatgtt

SEQ ID NO: 13 - DNA, 321 bp, Artificial Sequence; identical to SEQ ID NO: 12
  synthetic

SEQ ID NO: 14 - DNA, 5838 bp, Artificial Sequence
  synthetic
agcgcccaatacgcaaaccgcctctccccgcgcgttggccgattcattaatgcagctggcacgacaggtttcccgactggaaagcgggcagtgagcgcaacgcaattaatgtgagttagctcactcattaggcaccccaggctttacactttatgcttccggctcgtatgttgtgtggaattgtgagcggataacaatttcacacaggaaacagctatgaccatgattacgccagatttaattaaggctgcgcgctcgctcgctcactgaggccgcccgggcaaagcccgggcgtcgggcgacctttggtcgcccggcctcagtgagcgagcgagcgcgcagagagggagtggccaactccatcactaggggttccttgtagttaatgattaacccgccatgctacttatctacgtagccatgctctaggaagatcggaattcgcccttaagctagctagttattaatagtaatcaattacggggtcattagttcatagcccatatatggagttccgcgttacataacttacggtaaatggcccgcctggctgaccgcccaacgacccccgcccattgacgtcaataatgacgtatgttcccatagtaacgccaatagggactttccattgacgtcaatgggtggagtatttacggtaaactgcccacttggcagtacatcaagtgtatcatatgccaagtacgccccctattgacgtcaatgacggtaaatggcccgcctggcattatgcccagtacatgaccttatgggactttcctacttggcagtacatctacgtattagtcatcgctattaccatggtgatgcggttttggcagtacatcaatgggcgtggatagcggtttgactcacggggatttccaagtctccaccccattgacgtcaatgggagtttgttttggcaccaaaatcaacgggactttccaaaatgtcgtaacaactccgccccattgacgcaaatgggcggtaggcgtgtacggtgggaggtctatataagcagagctggtttagtgaaccgtcagatcctgcagaagttggtcgtgaggcactgggcaggtaagtatcaaggttacaagacaggtttaaggagaccaatagaaactgggcttgtcgagacagagaagactcttgcgtttctgataggcacctattggtcttactgacatccactttgcctttctctccacaggtgtccaggcggccgccatggtgagcaagggcgaggagctgttcaccggggtggtgcccatcctggtcgagctggacggcgacgtaaacggccacaagttcagcgtgtccggcgagggcgagggcgatgccacctacggcaagctgaccctgaagttcatctgcaccaccggcaagctgcccgtgccctggcccaccctcgtgaccaccctgacctacggcgtgcagtgcttcagccgctaccccgaccacatgaagcagcacgacttcttcaagtccgccatgcccgaaggctacgtccaggagcgcaccatcttcttcaaggacgacggcaactacaagacccgcgccgaggtgaagttcgagggcgacaccctggtgaaccgcatcgagctgaagggcatcgacttcaaggaggacggcaacatcctggggcacaagctggagtacaactacaacagccacaacgtctatatcatggccgacaagcagaagaacggcatcaaggtgaacttcaagatccgccacaacatcgaggacggcagcgtgcagctcgccgaccactaccagcagaacacccccatcggcgacggccccgtgctgctgcccgacaaccactacctgagcacccagtccgccctgagcaaagaccccaacgagaagcgcgatcacatggtcctgctggagttcgtgaccgccgccgggatcactctcggcatggacgagctgtacaagtaataagcttggatccaatcaacctctggattacaaaatttgtgaaagattgactggtattcttaactatgttgctccttttacgctatgtggatacgctgctttaatgcctttgtgctgcgctattgcttcccgtatggctttcattttctcctccttgtataaatcctggttgctgtctctttatgaggagttgtggcccgttgtcaggcaacgtggcgtggtgtgcactgtgtttgctgacgcaacccccactggttggggcattgccaccacctgtcagctcctttccgggactttcgctttccccctccctattgccacggcggaactcatcgccgcctgccttgcccgctgctggacaggggctcggctgttgggcactgacaattccgtggtgttgtcggggaagctgacgtcctttccttggctgctcgcctgtgttgccacctggattctgcgcgggacgtccttctgctacgtcccttcggccctcaatccagcggaccttccttcccgcggcctgctgccggctctgcggcctcttccgcgtcttcgagatcttctagaacccaccgacaatgctgaatgtttagcactcaccgacaatagtgaatgtttagcacccaccgacaatgctgaatgtttagcactcaccgacaatagtgaatgtttagcacccaccgacaatgctgaatgtttagcactcaccgacaatagtgaatgtttctagaacccaccgacaatgctgaatgtttagcactcaccgacaatagtgaatgtttagcacccaccgacaatgctgaatgtttagcactcaccgacaatagtgaatgtttagcacccaccgacaatgctgaatgtttagcactcaccgacaatagtgaatgttagatctgcctcgactgtgccttctagttgccagccatctgttgtttgcccctcccccgtgccttccttgaccctggaaggtgccactcccactgtcctttcctaataaaatgaggaaattgcatcgcattgtctgagtaggtgtcattctattctggggggtggggtggggcaggacagcaagggggaggattgggaagacaatagcaggcatgctggggactcgagttaagggcgaattcccgattaggatcttcctagagcatggctacgtagataagtagcatggcgggttaatcattaactacaaggaacccctagtgatggagttggccactccctctctgcgcgctcgctcgctcactgaggccgggcgaccaaaggtcgcccgacgcccgggctttgcccgggcggcctcagtgagcgagcgagcgcgcagccttaattaacctaattcactggccgtcgttttacaacgtcgtgactgggaaaaccctggcgttacccaacttaatcgccttgcagcacatccccctttcgccagctggcgtaatagcgaagaggcccgcaccgatcgcccttcccaacagttgcgcagcctgaatggcgaatgggacgcgccctgtagcggcgcattaagcgcggcgggtgtggtggttacgcgcagcgtgaccgctacacttgccagcgccctagcgcccgctcctttcgctttcttcccttcctttctcgccacgttcgccggctttccccgtcaagctctaaatcgggggctccctttagggttccgatttagtgctttacggcacctcgaccccaaaaaacttgattagggtgatggttcacgtagtgggccatcgccccgatagacggtttttcgccctttgacgctggagttcacgttcctcaatagtggactcttgttccaaactggaacaacactcaaccctatctcggtctattcttttgatttataagggatttttccgatttcggcctattggttaaaaaatgagctgatttaacaaaaatttaacgcgaattttaacaaaatattaacgtttataatttcaggtggcatctttcggggaaatgtgcgcggaacccctatttgtttatttttctaaatacattcaaatatgtatccgctcatgagacaataaccctgataaatgcttcaataatattgaaaaaggaagagtatgagtattcaacatttccgtgtcgcccttattcccttttttgcggcattttgccttcctgtttttgctcacccagaaacgctggtgaaagtaaaagatgctgaagatcagttgggtgcacgagtgggttacatcgaactggatctcaatagtggtaagatccttgagagttttcgccccgaagaacgttttccaatgatgagcacttttaaagttctgctatgtggcgcggtattatcccgtattgacgccgggcaagagcaactcggtcgccgcatacactattctcagaatgacttggttgagtactcaccagtcacagaaaagcatcttacggatggcatgacagtaagagaattatgcagtgctgccataaccatgagtgataacactgcggccaacttacttctgacaacgatcggaggaccgaaggagctaaccgcttttttgcacaacatgggggatcatgtaactcgccttgatcgttgggaaccggagctgaatgaagccataccaaacgacgagcgtgacaccacgatgcctgtagtaatggtaacaacgttgcgcaaactattaactggcgaactacttactctagcttcccggcaacaattaatagactggatggaggcggataaagttgcaggaccacttctgcgctcggcccttccggctggctggtttattgctgataaatctggagccggtgagcgtgggtctcgcggtatcattgcagcactggggccagatggtaagccctcccgtatcgtagttatctacacgacggggagtcaggcaactatggatgaacgaaatagacagatcgctgagataggtgcctcactgattaagcattggtaactgtcagaccaagtttactcatatatactttagattgatttaaaacttcatttttaatttaaaaggatctaggtgaagatcctttttgataatctcatgaccaaaatcccttaacgtgagttttcgttccactgagcgtcagaccccgtagaaaagatcaaaggatcttcttgagatcctttttttctgcgcgtaatctgctgcttgcaaacaaaaaaaccaccgctaccagcggtggtttgtttgccggatcaagagctaccaactctttttccgaaggtaactggcttcagcagagcgcagataccaaatactgtccttctagtgtagccgtagttaggccaccacttcaagaactctgtagcaccgcctacatacctcgctctgctaatcctgttaccagtggctgctgccagtggcgataagtcgtgtcttaccgggttggactcaagacgatagttaccggataaggcgcagcggtcgggctgaacggggggttcgtgcacacagcccagcttggagcgaacgacctacaccgaactgagatacctacagcgtgagctatgagaaagcgccacgcttcccgaagggagaaaggcggacaggtatccggtaagcggcagggtcggaacaggagagcgcacgagggagcttccagggggaaacgcctggtatctttatagtcctgtcgggtttcgccacctctgacttgagcgtcgatttttgtgatgctcgtcaggggggcggagcctatggaaaaacgccagcaacgcggcctttttacggttcctggccttttgctgcggttttgctcacatgttctttcctgcgttatcccctgattctgtggataaccgtattaccgcctttgagtgagctgataccgctcgccgcagccgaacgaccgagcgcagcgagtcagtgagcgaggaagcggaag

SEQ ID NO: 15 - DNA, 28 bp, Artificial Sequence
  synthetic
gctctagagacttctttctgcggaaatg

SEQ ID NO: 16 - DNA, 28 bp, Artificial Sequence
  synthetic
gctctagactgttttctatggccaggtg

SEQ ID NO: 17 - DNA, 36 bp, Artificial Sequence
  synthetic
ccacaggcagatgcgcgtcttgaaagctcccgggcc

SEQ ID NO: 18 - DNA, 36 bp, Artificial Sequence
  synthetic
ggcccgggagctttcaagacgcgcatctgcctgtgg

SEQ ID NO: 19 - DNA, 31 bp, Artificial Sequence
  synthetic
gctctagagcactacagatatcatattgagg

SEQ ID NO: 20 - DNA, 31 bp, Artificial Sequence
  synthetic
gctctagatagatttgaaacattcgtttccc

SEQ ID NO: 21 - DNA, 45 bp, Artificial Sequence
  synthetic
ctgagctaataaagggaaacgccggtttcaaatctctaggtcggg

SEQ ID NO: 22 - DNA, 45 bp, Artificial Sequence
  synthetic
cccgacctagagatttgaaaccggcgtttccctttattagctcag

SEQ ID NO: 23 - DNA, 28 bp, Artificial Sequence
  synthetic
gctctagagcctagctagaatatatgac

SEQ ID NO: 24 - DNA, 28 bp, Artificial Sequence
  synthetic
gctctagacacaggcttcctacatttag

SEQ ID NO: 25 - DNA, 36 bp, Artificial Sequence
  synthetic
caagtccatgcgcgttaaaatgtacaggtgggattg

SEQ ID NO: 26 - DNA, 36 bp, Artificial Sequence
  synthetic
caatcccacctgtacattttaacgcgcatggacttg

SEQ ID NO: 27 - DNA, 29 bp, Artificial Sequence
  synthetic
gctctagagccacctgcttctgactttag

SEQ ID NO: 28 - DNA, 28 bp, Artificial Sequence
  synthetic
gctctagacaacttcagtccttacattg

SEQ ID NO: 29 - DNA, 40 bp, Artificial Sequence
  synthetic
gaagataagttggttgggcgtctccagcactatgcatccc

SEQ ID NO: 30 - DNA, 40 bp, Artificial Sequence
  synthetic
gggatgcatagtgctggagacgcccaaccaacttatcttc

SEQ ID NO: 31 - DNA, 29 bp, Artificial Sequence
  synthetic
gctctagactgagagaagaaccacagttg

SEQ ID NO: 32 - DNA, 29 bp, Artificial Sequence
  synthetic
gctctagaccctggatttgataaatatcc

SEQ ID NO: 33 - DNA, 49 bp, Artificial Sequence
  synthetic
cggtcctgaaattttcatcttgccggtctttgtattaaactgaattttc

SEQ ID NO: 34 - DNA, 49 bp, Artificial Sequence
  synthetic
gaaaattcagtttaatacaaagaccggcaagatgaaaatttcaggaccg

SEQ ID NO: 35 - DNA, 40 bp, Artificial Sequence
  synthetic
gccgtgtaactcctgcaatgccggtttatgtgattgaagc

SEQ ID NO: 36 - DNA, 40 bp, Artificial Sequence
  synthetic
gcttcaatcacataaaccggcattgcaggagttacacggc

SEQ ID NO: 37 - DNA, 21 bp, Artificial Sequence
  synthetic
aacaccctttccaaatcctca

SEQ ID NO: 38 - DNA, 20 bp, Artificial Sequence
  synthetic
tggcgtcgtgattagtgatg

SEQ ID NO: 39 - DNA, 20 bp, Artificial Sequence
  synthetic
atgttcgtcatgggtgtgaa

SEQ ID NO: 40 - DNA, 20 bp, Artificial Sequence
  synthetic
aggggtgctaagcagttggt

SEQ ID NO: 41 - DNA, 20 bp, Artificial Sequence
  synthetic
gcttggccctctcagactct

SEQ ID NO: 42 - DNA, 20 bp, Artificial Sequence
  synthetic
gccactacagacaccgcacg

SEQ ID NO: 43 - DNA, 20 bp, Artificial Sequence
  synthetic
gagtgatgtccgcacagaag

SEQ ID NO: 44 - DNA, 20 bp, Artificial Sequence
  synthetic
gtttgcgtttgctgatcttc

SEQ ID NO: 45 - DNA, 20 bp, Artificial Sequence
  synthetic
gctgccgtacccctttatcg

SEQ ID NO: 46 - DNA, 20 bp, Artificial Sequence
  synthetic
cactggagacttgcatgcac

SEQ ID NO: 47 - DNA, 21 bp, Artificial Sequence
  synthetic
ggcgttttagcccaggtcttc

SEQ ID NO: 48 - DNA, 20 bp, Artificial Sequence
  synthetic
gctaccatctgcttcacaac

SEQ ID NO: 49 - DNA, 20 bp, Artificial Sequence
  synthetic
cccgagactacggtgtgctg

SEQ ID NO: 50 - DNA, 20 bp, Artificial Sequence
  synthetic
cactgggagatcgttgacgc

SEQ ID NO: 51 - DNA, 20 bp, Artificial Sequence
  synthetic
agcttgctggtgaaaaggac

SEQ ID NO: 52 - DNA, 20 bp, Artificial Sequence
  synthetic
gtcaagggcatatccacaac

SEQ ID NO: 53 - DNA, 20 bp, Artificial Sequence
  synthetic
ggtgctgagtatgtcgtgga

SEQ ID NO: 54 - DNA, 20 bp, Artificial Sequence
  synthetic
ctaagcagttggtggtgcag

SEQ ID NO: 55 - DNA, 20 bp, Artificial Sequence
  synthetic
acaacatcgccctgtggatg

SEQ ID NO: 56 - DNA, 20 bp, Artificial Sequence
  synthetic
gtttgtcgacctcacttgtg

SEQ ID NO: 57 - DNA, 21 bp, Artificial Sequence
  synthetic
gcttcatcgaaccattagcag

SEQ ID NO: 58 - DNA, 20 bp, Artificial Sequence
  synthetic
ccagcagcacatttctgatg

SEQ ID NO: 59 - DNA, 20 bp, Artificial Sequence
  synthetic
ggtcctgattgcagatcttg

SEQ ID NO: 60 - DNA, 19 bp, Artificial Sequence
  synthetic
gtcaactgcttctgcacac

SEQ ID NO: 61 - DNA, 21 bp, Artificial Sequence
  synthetic
gcctatatgtactgcttcatc

SEQ ID NO: 62 - DNA, 20 bp, Artificial Sequence
  synthetic
caacgtcaaatagctgactc

SEQ ID NO: 63 - DNA, 20 bp, Artificial Sequence
  synthetic
caccaacctctcgtacatcg

SEQ ID NO: 64 - DNA, 20 bp, Artificial Sequence
  synthetic
gtgcccggatgatgtcattg

SEQ ID NO: 65 - DNA, 20 bp, Artificial Sequence
  synthetic
ccatcaagaagaccaccaag

SEQ ID NO: 66 - DNA, 20 bp, Artificial Sequence
  synthetic
caagtgacatctctctctac

SEQ ID NO: 67 - DNA, 20 bp, Artificial Sequence
  synthetic
cttactggagtccaagatgc

SEQ ID NO: 68 - DNA, 20 bp, Artificial Sequence
  synthetic
ggagccaacagaatcctttc

SEQ ID NO: 69 - DNA, 20 bp, Artificial Sequence
  synthetic
gaatcctactgacaaaccag

SEQ ID NO: 70 - DNA, 20 bp, Artificial Sequence
  synthetic
gaggtcgacattcaccattc

SEQ ID NO: 71 - DNA, 20 bp, Artificial Sequence
  synthetic
gatgatcatggcagctcgga

SEQ ID NO: 72 - DNA, 20 bp, Artificial Sequence
  synthetic
ctcgcacagatctctttagg

SEQ ID NO: 73 - DNA, 21 bp, Artificial Sequence
  synthetic
ggagtatttctgcctcaacag

SEQ ID NO: 74 - DNA, 20 bp, Artificial Sequence
  synthetic
ctctccattgacaacagcag

SEQ ID NO: 75 - DNA, 21 bp, Artificial Sequence
  synthetic
ggaatgcaccgtaaaatctgc

SEQ ID NO: 76 - DNA, 20 bp, Artificial Sequence
  synthetic
ttctcaagagcagcgaaagc

SEQ ID NO: 77 - DNA, 19 bp, Artificial Sequence
  synthetic
ttcttttccctccgtgctc

SEQ ID NO: 78 - DNA, 20 bp, Artificial Sequence
  synthetic
ggatccgagtgtgaatttcc

SEQ ID NO: 79 - DNA, 23 bp, Artificial Sequence
  synthetic
ttatagagcgatacaagggggag

SEQ ID NO: 80 - DNA, 23 bp, Artificial Sequence
  synthetic
cgccgtctgattatcttgatgag

SEQ ID NO: 81 - DNA, 21 bp, Artificial Sequence
  synthetic
gccacacttggaggtgaaatc

SEQ ID NO: 82 - DNA, 19 bp, Artificial Sequence
  synthetic
aagcggaagttgctcatcg

SEQ ID NO: 83 - DNA, 20 bp, Artificial Sequence
  synthetic
tggacttacggcttgtcacc

SEQ ID NO: 84 - DNA, 20 bp, Artificial Sequence
  synthetic
aagcccggaactgcttattc

SEQ ID NO: 85 - DNA, 20 bp, Artificial Sequence
  synthetic
cagcaacagcaccaaaggtc

SEQ ID NO: 86 - DNA, 20 bp, Artificial Sequence
  synthetic
acagatgcaacgaccacaag

SEQ ID NO: 87 - DNA, 21 bp, Artificial Sequence
  synthetic
ggctcttagcacaattcttcg

SEQ ID NO: 88 - DNA, 19 bp, Artificial Sequence
  synthetic
gaatgcccccataggacac

SEQ ID NO: 89 - DNA, 21 bp, Artificial Sequence
  synthetic
ccctaactccacaaacacctg

SEQ ID NO: 90 - DNA, 20 bp, Artificial Sequence
  synthetic
atgacattgcccgttaggac

SEQ ID NO: 91 - DNA, 19 bp, Artificial Sequence
  synthetic
ctgaacaggaacagcgacc

SEQ ID NO: 92 - DNA, 20 bp, Artificial Sequence
  synthetic
tgaggagctccaataacgtc

SEQ ID NO: 93 - DNA, 20 bp, Artificial Sequence
  synthetic
cggcaagctgatagtcgatg

SEQ ID NO: 94 - DNA, 20 bp, Artificial Sequence
  synthetic
agaaacactccggtggactc

SEQ ID NO: 95 - DNA, 21 bp, Artificial Sequence
  synthetic
ggatgacggagtatttaaacg

SEQ ID NO: 96 - DNA, 20 bp, Artificial Sequence
  synthetic
ggccgaagacagtcttgatg

SEQ ID NO: 97 - DNA, 19 bp, Artificial Sequence
  synthetic
cgcgaaaagagtggtgaac

SEQ ID NO: 98 - DNA, 19 bp, Artificial Sequence
  synthetic
ccttcaaggactgacacac

SEQ ID NO: 99 - DNA, 20 bp, Artificial Sequence
  synthetic
cagatgacaaagacgtgctg

SEQ ID NO: 100 - DNA, 20 bp, Artificial Sequence
  synthetic
ctccacatcttctgtcctca

SEQ ID NO: 101 - DNA, 20 bp, Artificial Sequence
  synthetic
gcagcgacagcagatagttc

SEQ ID NO: 102 - DNA, 20 bp, Artificial Sequence
  synthetic
gccgagatgttgtccaacag

SEQ ID NO: 103 - DNA, 19 bp, Artificial Sequence
  synthetic
caccgacaaacccatcatc

SEQ ID NO: 104 - DNA, 19 bp, Artificial Sequence
  synthetic
gaattccgggtcgatgtag

SEQ ID NO: 105 - DNA, 19 bp, Artificial Sequence
  synthetic
gttctgcaaggccaaactg

SEQ ID NO: 106 - DNA, 19 bp, Artificial Sequence
  synthetic
cgtctccaagtggttgaag

SEQ ID NO: 107 - DNA, 19 bp, Artificial Sequence
  synthetic
gtcctgttcttctaccctc

SEQ ID NO: 108 - DNA, 20 bp, Artificial Sequence
  synthetic
agtgagaatccacagacacc

SEQ ID NO: 109 - DNA, 20 bp, Artificial Sequence
  synthetic
ggacggattgccttcatttg

SEQ ID NO: 110 - DNA, 19 bp, Artificial Sequence
  synthetic
gtttgcaggtgccagaagg

SEQ ID NO: 111 - DNA, 25 bp, Artificial Sequence
  synthetic
aactcaccgacagcgttgaatgttc

SEQ ID NO: 112 - DNA, 25 bp, Artificial Sequence
  synthetic
aacccaccgacagcaatgaatgttg

SEQ ID NO: 113 - DNA, 23 bp, Artificial Sequence
  synthetic
  misc_feature 12..12: /note="n is A, C or T"
  misc_feature 13..13: /note="n is A, G or T"
  misc_feature 14..14: /note="n is A, C or T"
  misc_feature 15..15: /note="n is A, C or G"
actcaccgacannnntgaatgtt

SEQ ID NO: 114 - DNA, 23 bp, Artificial Sequence
  synthetic
  misc_feature 12..12: /note="n is A, C or T"
  misc_feature 13..13: /note="n is A, G or T"
  misc_feature 14..15: /note="n is C, G or T"
acccaccgacannnntgaatgtt